European Patent Specification EP 4 047 011 B1, published July 2, 2025. Title: HYBRID ANTIMICROBIAL PROTEIN HAVING STRONG BACTERICIDAL EFFECT AND APPLICATION THEREOF. Applicant: Jiangxi Yuansheng Biological Technology Co., Ltd. The sequence listing filed with the application follows.

SEQUENCE LISTING (12 sequences)

SEQ ID NO: 1 - protein, 285 aa, Artificial Sequence
MAILTKDGFGIIRNELFGGKLDQTQVDAINFIVEKATESGLSYPEAAYLLATIYHETGLPSGYRTMQPIKEAGSDNYLRSKKYYPYIGYGYVQLTWKENYGRIGKLIGIDLIKNPEKALEPLIAIQIAIKGMLNGWFTGVGFRRKRPVSKYNKQQYIAARNIINGKDKAELIAKYAIIFERALRSLGSNSTSNSSTNSGSTGKVSLPNRVIRVTKPIVHGSDVLAIQKALSSLYFYPEKGAKDNGSDSYYGPKTANAVKRFQSVNGLVADGVYGPKTRAAILKKL

SEQ ID NO: 2 - DNA, 864 bp, Artificial Sequence
ccatggctatcctgaccaaagatggctttggcatcattcgcaacgaactgtttggcggcaaactggatcagacacaggtggatgccattaattttattgttgaaaaagctaccgaatctgggttaagttatccggaagcggcctatctgttagcgacgatctatcatgaaacgggtctgccgagcggttatcgtaccatgcagccaatcaaagaagccggtagtgataattacctccgctctaaaaaatattatccgtatatcggctatggctatgttcagctgacgtggaaagaaaattatggtcgtattggtaaactgatcggcatcgacttgatcaaaaatccggaaaaagccttagaaccgctgattgcgattcagattgccatcaaaggtatgctgaatggttggtttacaggtgtgggctttcgtcgcaaacgtccagtgagtaaatataacaagcagcagtatattgctgcacgcaatatcattaatggtaaagataaagcagaactgatcgcgaaatatgccatcatctttgaacgcgccctgcgttctctgggctccaatagtacctctaatagtagcaccaattcaggctctaccggtaaagtgagtctgccgaatcgtgtgattcgcgtgaccaaaccgattgttcatggtagcgatgtgctggcaattcagaaagcactgtcaagcctgtatttttatccggaaaaaggtgccaaagataatggttccgatagctattatggtccgaaaaccgccaatgccgttaaacgctttcagtctgttaatggcttagttgcagatggcgtgtatggcccgaaaacccgcgcagccattctgaaaaaactgtaagctt

SEQ ID NO: 3 - protein, 285 aa, Artificial Sequence
MALITKDGFSIIRNELFNGKLDQTQVDAINFLVEKSTEYGLTYPEAAYLLGTIYHETALPSAYRTMQPIKEAGSDSYLKSKKYYPYIGYGYVQLTWEDNYERIGKLIGIDLVKNPEKALEPLISIQIAIKGMLNGWFTAVRITRKRPVAKYNKQPYVAARNIINGKDRAELIPNYAFIFEKARRLIGSNSTSNSSTNSGSTGKVSLPNRVIRVTKPIVHGSDVLAIQKALSSLYFYPEKGAKDNGSDSYYGPKTANAVKRFQSVNGLVADGVYGPKTRAAILKKL

SEQ ID NO: 4 - DNA, 864 bp, Artificial Sequence
ccatggctctgatcaccaaagatggctttagtatcattcgcaacgaactgtttaatggcaaactggatcagacacaggtggatgccattaattttctggttgaaaaatctaccgaatatgggttaacgtatccggaagcggcctatctgttaggtacgatctatcatgaaacggctctgccgagcgcttatcgtaccatgcagccaatcaaagaagccggtagtgatagttacctcaaatctaaaaaatattatccgtatatcggctatggctatgttcagctgacgtgggaagataattatgaacgtattggtaaactgatcggcatcgacttggttaaaaatccggaaaaagccttagaaccgctgattagtattcagattgccatcaaaggtatgctgaatggttggtttacagctgtgcgtatcacccgcaaacgtccagtggctaaatataacaagcagccgtatgttgctgcacgcaatatcattaatggtaaagatcgtgcagaactgatcccgaattatgcctttatctttgaaaaagcccgccgtctgatcggctccaatagtacctctaatagtagcaccaattcaggctctaccggtaaagtgagtctgccgaatcgtgtgattcgcgtgaccaaaccgattgttcatggtagcgatgtgctggcaattcagaaagcactgtcaagcctgtatttttatccggaaaaaggtgccaaagataatggttccgatagctattatggtccgaaaaccgccaatgccgttaaacgctttcagtctgttaatggcttagttgcagatggcgtgtatggcccgaaaacccgcgcagccattctgaaaaaactgtaagctt

SEQ ID NO: 5 - protein, 285 aa, Artificial Sequence
MAILTKDGFGIIRNELFGGKLDQTQVDAINFIVEKATESGLSYPEAAYLLATIYHETGLPSGYRTMQPIKEAGSDNYLRSKKYYPYIGYGYVQLTWKENYGRIGKLIGIDLIKNPEKALEPLIAIQIAIKGMLNGWFTGVGFRRKRPVSKYNKQQYIAARNIINGKDKAELIAKYAIIFERALRSLGSNSTSNSSTNSGSTGKVTLPSGVIRVTKPMVHGDDVLAIQKALAALYFYPDKGAKDNGIDGVYGPKTANAVKRFQSVNGLTADGIYGPKTRAAIEEKL

SEQ ID NO: 6 - DNA, 864 bp, Artificial Sequence
ccatggctatcctgaccaaagatggctttggcatcattcgcaacgaactgtttggcggcaaactggatcagacacaggtggatgccattaattttattgttgaaaaagctaccgaatctgggttaagttatccggaagcggcctatctgttagcgacgatctatcatgaaacgggtctgccgagcggttatcgtaccatgcagccaatcaaagaagccggtagtgataattacctccgctctaaaaaatattatccgtatatcggctatggctatgttcagctgacgtggaaagaaaattatggtcgtattggtaaactgatcggcatcgacttgatcaaaaatccggaaaaagccttagaaccgctgattgcgattcagattgccatcaaaggtatgctgaatggttggtttacaggtgtgggctttcgtcgcaaacgtccagtgagtaaatataacaagcagcagtatattgctgcacgcaatatcattaatggtaaagataaagcagaactgatcgcgaaatatgccatcatctttgaacgcgccctgcgttctctgggctccaatagtacctctaatagtagcaccaattcaggctctaccggtaaagtgacactgccgagtggtgtgattcgcgtgaccaaaccgatggttcatggtgacgatgtgctggcaattcagaaagcactggcagccctgtatttttatccggataaaggtgccaaagataatggtattgatggtgtttatggtccgaaaaccgccaatgccgttaaacgctttcagtctgttaatggcttaacagcagatggcatttatggcccgaaaacccgcgcagccattgaagaaaaactgtaagctt

SEQ ID NO: 7 - protein, 285 aa, Artificial Sequence
MAKVSLPNRVIRVTKPIVHGSDVLAIQKALSSLYFYPEKGAKDNGSDSYYGPKTANAVKRFQSVNGLVADGVYGPKTRAAILKKLGSNSTSNSSTNSGSTGILTKDGFGIIRNELFGGKLDQTQVDAINFIVEKATESGLSYPEAAYLLATIYHETGLPSGYRTMQPIKEAGSDNYLRSKKYYPYIGYGYVQLTWKENYGRIGKLIGIDLIKNPEKALEPLIAIQIAIKGMLNGWFTGVGFRRKRPVSKYNKQQYIAARNIINGKDKAELIAKYAIIFERALRSL

SEQ ID NO: 8 - DNA, 864 bp, Artificial Sequence
ccatggctaaagtgagtctgccgaatcgtgtgattcgcgtgaccaaaccgattgttcatggtagcgatgtgctggcaattcagaaagcactgtcaagcctgtatttttatccggaaaaaggtgccaaagataatggttccgatagctattatggtccgaaaaccgccaatgccgttaaacgctttcagtctgttaatggcttagttgcagatggcgtgtatggcccgaaaacccgcgcagccattctgaaaaaactgggctccaatagtacctctaatagtagcaccaattcaggctctaccggtatcctgaccaaagatggctttggcatcattcgcaacgaactgtttggcggcaaactggatcagacacaggtggatgccattaattttattgttgaaaaagctaccgaatctgggttaagttatccggaagcggcctatctgttagcgacgatctatcatgaaacgggtctgccgagcggttatcgtaccatgcagccaatcaaagaagccggtagtgataattacctccgctctaaaaaatattatccgtatatcggctatggctatgttcagctgacgtggaaagaaaattatggtcgtattggtaaactgatcggcatcgacttgatcaaaaatccggaaaaagccttagaaccgctgattgcgattcagattgccatcaaaggtatgctgaatggttggtttacaggtgtgggctttcgtcgcaaacgtccagtgagtaaatataacaagcagcagtatattgctgcacgcaatatcattaatggtaaagataaagcagaactgatcgcgaaatatgccatcatctttgaacgcgccctgcgttctctgtaagctt

SEQ ID NO: 9 - protein, 186 aa, AB46 1-185 aa
MAILTKDGFGIIRNELFGGKLDQTQVDAINFIVEKATESGLSYPEAAYLLATIYHETGLPSGYRTMQPIKEAGSDNYLRSKKYYPYIGYGYVQLTWKENYGRIGKLIGIDLIKNPEKALEPLIAIQIAIKGMLNGWFTGVGFRRKRPVSKYNKQQYIAARNIINGKDKAELIAKYAIIFERALRSL

SEQ ID NO: 10 - protein, 185 aa, Artificial Sequence
MLITKDGFSIIRNELFNGKLDQTQVDAINFLVEKSTEYGLTYPEAAYLLGTIYHETALPSAYRTMQPIKEAGSDSYLKSKKYYPYIGYGYVQLTWEDNYERIGKLIGIDLVKNPEKALEPLISIQIAIKGMLNGWFTAVRITRKRPVAKYNKQPYVAARNIINGKDRAELIPNYAFIFEKARRLI

SEQ ID NO: 11 - protein, 83 aa, SP10 154-236 aa
KVSLPNRVIRVTKPIVHGSDVLAIQKALSSLYFYPEKGAKDNGSDSYYGPKTANAVKRFQSVNGLVADGVYGPKTRAAILKKL

SEQ ID NO: 12 - protein, 83 aa, Artificial Sequence
KVTLPSGVIRVTKPMVHGDDVLAIQKALAALYFYPDKGAKDNGIDGVYGPKTANAVKRFQSVNGLTADGIYGPKTRAAIEEKL